European Patent Specification EP 3 662 073 B1, published May 22, 2024. Title: Microorganism and method for improved 1,3-propanediol production by fermentation on a culture medium with high glycerine content. Applicant: METABOLIC EXPLORER. The sequence listing filed with the application follows.

SEQUENCE LISTING (25 sequences)

SEQ ID NO: 1 - DNA, 690 bp, Clostridium acetobutylicum
  misc_feature: CA_C0884 gene sequence
atggataaaaaaattttaaccgtattaaaacattgtatcttattttcaaaaattgaaactcaggaaattgatcatttattttcatctataaattactcaataaaagaatactataaagatgaaactatcgcaattgaaggcgatacgtgcaataaaattggaatagtattaagcggttgtgttgaaatacagaaaatttacgaatctggtaaaagtcttacaataacaacactagaagaaagcaagatatttggtgaagcaataatattctccaataaaacaagctatccttctacaataatagcatgtactaaaagtactataatttttattcccaaagcctcaatatctaaattatgcagcgacaattcccttttccttaatggctttatgtctcttctatctaataagatattgatgttgaataaaaaattaaaaaatatgtcttatcatactataagagagaaaatatcaaactatatacttgaacagtacgaagctcaaaataacttaacttttaaaatgaataagtcaaaaaaacagttgtctgaaatgcttggaattccaaggccatcattatctagagaattcataaacctacgtgaagaaggaattatagactttgatagaacatctattacaatattagatattaactctttaaaagaaattttagaagctgcagaataa

SEQ ID NO: 2 - protein, 229 aa, Clostridium acetobutylicum
  MISC_FEATURE: CA_C0884 protein sequence : NP_347520.1
MDKKILTVLKHCILFSKIETQEIDHLFSSINYSIKEYYKDETIAIEGDTCNKIGIVLSGCVEIQKIYESGKSLTITTLEESKIFGEAIIFSNKTSYPSTIIACTKSTIIFIPKASISKLCSDNSLFLNGFMSLLSNKILMLNKKLKNMSYHTIREKISNYILEQYEAQNNLTFKMNKSKKQLSEMLGIPRPSLSREFINLREEGIIDFDRTSITILDINSLKEILEAAE

SEQ ID NO: 3 - DNA, 711 bp, Clostridium acetobutylicum
  misc_feature: CA_C0885 gene sequence
atgaaaagaaaaatagtaaacatagataaagataaatgtaatggatgtggactttgtagtgaagcatgtcatgaaaatgcaattgaaataattaatggaaaagcagagcttttatctgatgaatattgtgatggtttaggagattgtttacctcattgtccagttgatgcaataactataatagagagagaaagtaaggaatatgatgaagaggcagttcagagaagaattgaagaaaagaaaaaatcaaagttagctaaaccctgtggatgtccaggagctatggctaaaaaaatagaaagagtagctaagcctttagctaaagtaaaggaagataggtcttctgtttcagagttaatgcagtggccagttcagttaaggcttgtaagtccaggagctccatattttaaaaatgctaatcttttagtagctgcagattgtacagcctatgcttatggtgactttcacaatgattttataaagaatcatataacagtaataggatgtccaaaacttgatgatgttacatattacaaagataagttgaaagaaattatagaacttaatgaccttaagagtataacagttgttagaatggaggtaccttgctgttcaggcatagtttcagcagtaaagactgctatgcttgaagcaaaagttatagtaccttttagagaagttattataggaactaatggtgaaattagataa

SEQ ID NO: 4 - protein, 236 aa, Clostridium acetobutylicum
  MISC_FEATURE: CA_C0885 protein sequence : NP_347521.1
MKRKIVNIDKDKCNGCGLCSEACHENAIEIINGKAELLSDEYCDGLGDCLPHCPVDAITIIERESKEYDEEAVQRRIEEKKKSKLAKPCGCPGAMAKKIERVAKPLAKVKEDRSSVSELMQWPVQLRLVSPGAPYFKNANLLVAADCTAYAYGDFHNDFIKNHITVIGCPKLDDVTYYKDKLKEIIELNDLKSITVVRMEVPCCSGIVSAVKTAMLEAKVIVPFREVIIGTNGEIR

SEQ ID NO: 5 - DNA, 684 bp, Clostridium pasteurianum
  misc_feature: BEE63_RS05095 gene sequence
atggataaagaacttttaagtatattaaagaactgtattttattttgcaaaattgatgatactaaaattaatgagcttttttcatatataaattattcaataaaaaaatactcaaatggagaaactgtggccattgaaggtgacgagtgcagcagcataggtataattttagacggttttgctgagatacaaaaaatctacgaatccggcaaaagtttaactatagagaccttaaacactaacaagatatttggtgaagcaataatattttctaaaaaaaatacttatccggctacaataatttcatgtgccaaaacaagtatattattcataccaaaatcctcaataattaaattatgcagcgaaaattcaaattttctaaacggctttatgtctcttctatctaataaaatattaatgctaaataaaaagttaaaaaatctttcatataacacaattagagaaaaagtagcaaattacctacttgaagagactataatccaaaaaaatccaaatataaaaatgaataaatcaaaaaaacagctgtctgaattactcggtattccacgtccttctctgtctagagaattaataaagttaaggaacgatggtatcatttcctttgatagaaattatattaaaatattaaatatggatgagttaaaaaatatcctagataagtag

SEQ ID NO: 6 - protein, 227 aa, Clostridium pasteurianum
  MISC_FEATURE: BEE63_RS05095 protein sequence : WP_066020350
MDKELLSILKNCILFCKIDDTKINELFSYINYSIKKYSNGETVAIEGDECSSIGIILDGFAEIQKIYESGKSLTIETLNTNKIFGEAIIFSKKNTYPATIISCAKTSILFIPKSSIIKLCSENSNFLNGFMSLLSNKILMLNKKLKNLSYNTIREKVANYLLEETIIQKNPNIKMNKSKKQLSELLGIPRPSLSRELIKLRNDGIISFDRNYIKILNMDELKNILDK

SEQ ID NO: 7 - DNA, 690 bp, Clostridium butyricum
  misc_feature: CBY_RS14495 gene sequence
atgaaaaatgttaatgagattatagataaaataaagcaaaatgaattttttaaggggatagatgataaaaaaatagaaatgattatttcagaattaagtcatatttctaaggaatattcaaaaggacaggtaattgctaatgagggggaggtttgtaaaaatctaggattagtcgtagatggaattgttgagatacagagaatatactcaagcggaaaacatatagttcttaaacgtatgggagcaggagaagtttttggagaagccataatattttcagataaaaataaatatccagccacaataattgcttcttcggattgtataatatcttatttgaaaaaagaagatattattaaactttgccttaatgaagaaataatcttaaagaattttataactttattgagcaataaaatttttatattaaatagaaaaataaaaaccatatcttttaaaacaatacgacagaaagttgttaactttatattagaacagtcaaaaagtcagaacaataaaactgtaattttgaaaataagtaaagagcagatagcatctttacttggaatacctagaccatcactttcaagagagcttatgaagcttagagatgatggacttattgaatttgataggaacaaaataagtattataaatatagaaagacttgaagaagaacttttagaatag

SEQ ID NO: 8 - protein, 229 aa, Clostridium butyricum
  MISC_FEATURE: CBY_RS14495 protein sequence : WP_003410673.1
MKNVNEIIDKIKQNEFFKGIDDKKIEMIISELSHISKEYSKGQVIANEGEVCKNLGLVVDGIVEIQRIYSSGKHIVLKRMGAGEVFGEAIIFSDKNKYPATIIASSDCIISYLKKEDIIKLCLNEEIILKNFITLLSNKIFILNRKIKTISFKTIRQKVVNFILEQSKSQNNKTVILKISKEQIASLLGIPRPSLSRELMKLRDDGLIEFDRNKISIINIERLEEELLE

SEQ ID NO: 9 - DNA, 690 bp, Clostridium butyricum
  misc_feature: K670_RS19640 gene sequence
atgaaaaatgctaatgagattatagataaaataaagcaaaatgaattttttaaggggatagatgataaaaaaatagaaatgattatttcagaattaagtcatatttctaaggaatattcaaaaggacaggtaattgctaatgagggggaggtttgtaaaaatctaggattagtcgtagatggaattgttgagatacagagaatatactcaagcggaaaacatatagttcttaaacgtatgggagcaggagaagtttttggagaagccataatattttcagataaaaataaatatccagccacaataattgcttcttcggattgtataatatcttatttgaaaaaagaagatattattaaactttgccttaatgaagaaataattttaaagaattttataactttattgagcaataaaatttttatattaaatagaaaaataaaaaccatatcttttaaaacaatacgacagaaagttgttaactttatattagaacagtcaaaaagtcagaacaataaaactgtaattttgaaaataagtaaagagcagatagcatctttacttggaatacctagaccatcactttcaagagagcttatgaaacttagagatgatggacttattgaatttgataggaacaaaataagtattataaatatagaaagacttgaagaagaacttttagaatag

SEQ ID NO: 10 - protein, 229 aa, Clostridium butyricum
  MISC_FEATURE: K670_RS19640 protein sequence : WP_035765453.1
MKNANEIIDKIKQNEFFKGIDDKKIEMIISELSHISKEYSKGQVIANEGEVCKNLGLVVDGIVEIQRIYSSGKHIVLKRMGAGEVFGEAIIFSDKNKYPATIIASSDCIISYLKKEDIIKLCLNEEIILKNFITLLSNKIFILNRKIKTISFKTIRQKVVNFILEQSKSQNNKTVILKISKEQIASLLGIPRPSLSRELMKLRDDGLIEFDRNKISIINIERLEEELLE

SEQ ID NO: 11 - DNA, 690 bp, Clostridium butyricum
  misc_feature: AT697_RS15885 gene sequence
atgaaaaatgttaatgagattatagataaaataaagcaaaatgaattttttaaggggatagatgataaaaaaatagaaatgattatttcagaattaagtcatatttataaggaatattcaaaaggacaggtaattgctaatgagggggaggtttgtaaaaatctaggattagtcgtagatggaattgttgagatacagagaatatactcaagcggaaaacatatagttcttaaacgtatgggagcaggagaagtttttggagaagccataatattttcagataaaaataaatatccagccacaataattgcttcttcggattgtataatatcttatttgaaaaaagaagatattattaaactttgccttaatgaagaaataatcttaaagaattttataactttattgagcaataaaatttttatattaaatagaaaaataaaaaccatatcttttaaaacaatacgacagaaagttgttaactttatattagaacagtcaaaaagtcagaacaataaaactgtaattttgaaaataagtaaagagcagatagcatctttacttggaatacctagaccatcactttcaagagagcttatgaagcttagagatgatggacttattgaatttgataggaacaaaataagtattataaatatagaaagacttgaagaagagcttttagaatag

SEQ ID NO: 12 - protein, 229 aa, Clostridium butyricum
  MISC_FEATURE: AT697_RS15885 protein sequence : WP_046057470.1
MKNVNEIIDKIKQNEFFKGIDDKKIEMIISELSHIYKEYSKGQVIANEGEVCKNLGLVVDGIVEIQRIYSSGKHIVLKRMGAGEVFGEAIIFSDKNKYPATIIASSDCIISYLKKEDIIKLCLNEEIILKNFITLLSNKIFILNRKIKTISFKTIRQKVVNFILEQSKSQNNKTVILKISKEQIASLLGIPRPSLSRELMKLRDDGLIEFDRNKISIINIERLEEELLE

SEQ ID NO: 13 - DNA, 711 bp, Clostridium pasteurianum
  misc_feature: BEE63_RS05090 gene sequence
atgaaaagaaaaatagtgaatatagataaagaaaaatgtaatggatgtggactttgtagtaaggcatgccatgaaaatgctatagaaataattgatggaaaagcagaacttgtttcggatgaatattgtgatggacttggagattgccttccacattgtccagaaaacgctataactataatagaaagagaaagtaaagaatacgatgaagaagctgtaaaaagaagaattgaaagtaaagaaaagaaaatgccatgtggatgtccaggttcaatggcaaaaaagataactagagtttctaaaaaagtagaagttaaacatgaagatacgggtgcagcatcagaacttatgcagtggcctgtacaattgcaattagtaaatccaaatgcaagctattttgaaggcgcaaatcttttagttgcagcggattgtacagcttatgcttatggtaactttcatcaagattttataaaaaatcatataactgtaataggttgtcctaaacttgacgatgttgagtactataagaataaaatcaaagaaattatagaaaataataatcttaaaagtattacagttaccagaatggaagtaccatgctgtggcggtatagtgtcagctgtaaagaatgctatgcttgaggcacaggttatattaccttatagagaagtagttataggaactaatggagaagtgaaggaagcgaagtaa

SEQ ID NO: 14 - protein, 236 aa, Clostridium pasteurianum
  MISC_FEATURE: BEE63_RS05090 protein sequence : WP_066020349.1
MKRKIVNIDKEKCNGCGLCSKACHENAIEIIDGKAELVSDEYCDGLGDCLPHCPENAITIIERESKEYDEEAVKRRIESKEKKMPCGCPGSMAKKITRVSKKVEVKHEDTGAASELMQWPVQLQLVNPNASYFEGANLLVAADCTAYAYGNFHQDFIKNHITVIGCPKLDDVEYYKNKIKEIIENNNLKSITVTRMEVPCCGGIVSAVKNAMLEAQVILPYREVVIGTNGEVKEAK

SEQ ID NO: 15 - DNA, 1524 bp, Clostridium acetobutylicum
  misc_feature: Full sequence comprising CA_C0884, the intergenic region, and CA_C0885
ttattctgcagcttctaaaatttcttttaaagagttaatatctaatattgtaatagatgttctatcaaagtctataattccttcttcacgtaggtttatgaattctctagataatgatggccttggaattccaagcatttcagacaactgtttttttgacttattcattttaaaagttaagttattttgagcttcgtactgttcaagtatatagtttgatattttctctcttatagtatgataagacatattttttaattttttattcaacatcaatatcttattagatagaagagacataaagccattaaggaaaagggaattgtcgctgcataatttagatattgaggctttgggaataaaaattatagtacttttagtacatgctattattgtagaaggatagcttgttttattggagaatattattgcttcaccaaatatcttgctttcttctagtgttgttattgtaagacttttaccagattcgtaaattttctgtatttcaacacaaccgcttaatactattccaattttattgcacgtatcgccttcaattgcgatagtttcatctttatagtattcttttattgagtaatttatagatgaaaataaatgatcaatttcctgagtttcaatttttgaaaataagatacaatgttttaatacggttaaaatttttttatccatgtttttctcccaatacttttttgtgtaacatatgttactgatatatttatataattttaatataatttaatcataaagacaagtaattttattttgcggaactttatatttaggaggaaaaaaatgaaaagaaaaatagtaaacatagataaagataaatgtaatggatgtggactttgtagtgaagcatgtcatgaaaatgcaattgaaataattaatggaaaagcagagcttttatctgatgaatattgtgatggtttaggagattgtttacctcattgtccagttgatgcaataactataatagagagagaaagtaaggaatatgatgaagaggcagttcagagaagaattgaagaaaagaaaaaatcaaagttagctaaaccctgtggatgtccaggagctatggctaaaaaaatagaaagagtagctaagcctttagctaaagtaaaggaagataggtcttctgtttcagagttaatgcagtggccagttcagttaaggcttgtaagtccaggagctccatattttaaaaatgctaatcttttagtagctgcagattgtacagcctatgcttatggtgactttcacaatgattttataaagaatcatataacagtaataggatgtccaaaacttgatgatgttacatattacaaagataagttgaaagaaattatagaacttaatgaccttaagagtataacagttgttagaatggaggtaccttgctgttcaggcatagtttcagcagtaaagactgctatgcttgaagcaaaagttatagtaccttttagagaagttattataggaactaatggtgaaattagataa

SEQ ID NO: 16 - DNA, 123 bp, Clostridium acetobutylicum
  misc_feature: Intergenic region between positions 1014117 and 1014239 of the C. acetobutylicum ATCC 824 genome
gtttttctcccaatacttttttgtgtaacatatgttactgatatatttatataattttaatataatttaatcataaagacaagtaattttattttgcggaactttatatttaggaggaaaaaa

SEQ ID NO: 17 - DNA, 124 bp, Artificial
  Intergenic region comprising a single nucleotide insertion
gtttttctcccaatacttttttgtgtaacatatgttactgatatatttatataattttaatataatttaatcataaagacaagtaattttattttgcggaactttatatttaggaggaaaaaaa

SEQ ID NO: 18 - DNA, 17 bp, Artificial
  Intergenic region forward primer
gccattaaggaaaaggg

SEQ ID NO: 19 - DNA, 19 bp, Artificial
  Intergenic region reverse primer
gctcctggacttacaagcc

SEQ ID NO: 20 - DNA, 20 bp, Artificial
  CA_C0884 gene based forward primer
gaagagacataaagccatta

SEQ ID NO: 21 - DNA, 21 bp, Artificial
  CA_C0884 gene based reverse primer
acaataacaacactagaagaa

SEQ ID NO: 22 - DNA, 19 bp, Artificial
  CA_C0885 gene based forward primer
gctaaaccctgtggatgtc

SEQ ID NO: 23 - DNA, 22 bp, Artificial
  CA_C0885 gene based reverse primer
ggacttacaagccttaactgaa

SEQ ID NO: 24 - DNA, 18 bp, Artificial
  CA_C1628 gene based forward primer
cccttagaggaggctatg

SEQ ID NO: 25 - DNA, 18 bp, Artificial
  CA_C1628 gene based reverse primer
gccatctcttacatctgg